European Patent Specification EP 2 968 536 B1, published June 28, 2023. Title: METHODS FOR MODULATING CHEMOTHERAPEUTIC CYTOTOXICITY. Applicant: The United States of America, as represented by the Secretary, Department of Health and Human Services Roberts, David D. Soto Pantoja, David R. The sequence listing filed with the application follows.

SEQUENCE LISTING (3 sequences)

SEQ ID NO: 1 - protein, 11 aa, Artificial Sequence
  Thrombospondin 1-derived CD47 binding peptide
FIRVVMYEGKK

SEQ ID NO: 2 - protein, 8 aa, Artificial Sequence
  CD47 binding peptide
RFYVVMWK

SEQ ID NO: 3 - DNA, 25 bp, Artificial Sequence
  CD47 antisense morpholino oligonucleotide
cgtcacaggcaggacccactgccca